European Patent Application EP 4 446 432 A1, published October 16, 2024. Title: Method for forming single-stranded DNA and mutant detection using same. Applicant: POSTECH Research and Business Development Foundation. The sequence listing filed with the application follows.

SEQUENCE LISTING (66 sequences)

SEQ ID NO: 1 - DNA, 82 bp, synthetic construct
  source 1..82: mol_type = other DNA
  misc_binding 1: bound_moiety = phosphate
ttcaaggctccctcagttgcccctatagtgagtcgtattaatttcgcgacaacacgcgaaattaatacgactcactataggg

SEQ ID NO: 2 - DNA, 62 bp, synthetic construct
  source 1..62: mol_type = other DNA
ggatccattcgttacctggctctcgccagtcgggatccgtgccaatgtgatcttttggtgta

SEQ ID NO: 3 - DNA, 222 bp, Severe acute respiratory syndrome coronavirus 2
  source 1..222: mol_type = genomic DNA
  primer_bind 1..19: note = SARS-CoV-2 PCR primer 1 binding region
  misc_binding 19..38: bound_moiety = Binding region of promoter probe for detecting target sequence of SARS-CoV-2
  misc_binding 39..55: bound_moiety = Binding region of reporter probe for detecting target sequence of SARS-CoV-2
  primer_bind 201..222: note = SARS-CoV-2 PCR primer 2 binding region
gacggcatcatatgggttgcaactgagggagccttgaatacaccaaaagatcacattggcacccgcaatcctgctaacaatgctgcaatcgtgctacaacttcctcaaggaacaacattgccaaaaggcttctacgcagaagggagcagaggcggcagtcaagcctcttctcgttcctcatcacgtagtcgcaacagttcaagaaattcaactccaggcagc

SEQ ID NO: 4 - DNA, 19 bp, synthetic construct
  source 1..19: mol_type = other DNA
gacggcatcatatgggttg

SEQ ID NO: 5 - DNA, 22 bp, synthetic construct
  source 1..22: mol_type = other DNA
gctgcctggagttgaatttctt

SEQ ID NO: 6 - DNA, 30 bp, synthetic construct
  source 1..30: mol_type = other DNA
caatgttgttccttgaggaagttgtagcac

SEQ ID NO: 7 - DNA, 40 bp, synthetic construct
  source 1..40: mol_type = other DNA
caatgttgttccttgaggaagttgtagcacgattgcagca

SEQ ID NO: 8 - DNA, 84 bp, synthetic construct
  source 1..84: mol_type = other DNA
  misc_binding 1: bound_moiety = Phosphate
gtgcatttcgctgattttggggccctatagtgagtcgtattaatttcgcgacaacacgcgaaattaatacgactcactataggg

SEQ ID NO: 9 - DNA, 59 bp, synthetic construct
  source 1..59: mol_type = other DNA
ggatccattcgttacctggctctcgccagtcgggatccgtccaccaaacgtaatgcgga

SEQ ID NO: 10 - DNA, 50 bp, synthetic construct
  source 1..50: mol_type = other DNA
ggggccgacgttgttttgatcgcgccccaccattctggttactgccagtt

SEQ ID NO: 11 - DNA, 10 bp, synthetic construct
  source 1..10: mol_type = other DNA
tatcagacat

SEQ ID NO: 12 - DNA, 130 bp, Severe acute respiratory syndrome coronavirus 2
  source 1..130: mol_type = genomic DNA
  primer_bind 14..33: note = Omicron PCR primer 1 binding region
  misc_binding 16..37: bound_moiety = Binding region of promoter probe for detecting target sequence of Omicron variant of SARS-CoV-2
  misc_binding 38..58: bound_moiety = Binding region of reporter probe for detecting target sequence of Omicron variant of SARS-CoV-2
  primer_bind 114..130: note = Omicron PCR primer 2 binding region
atgtctgataatggaccccaaaatcagcgaaatgcactccgcattacgtttggtggaccctcagattcaactggcagtaaccagaatggtggggcgcgatcaaaacaacgtcggccccaaggtttaccca

SEQ ID NO: 13 - DNA, 20 bp, synthetic construct
  source 1..20: mol_type = other DNA
gaccccaaaatcagcgaaat

SEQ ID NO: 14 - DNA, 17 bp, synthetic construct
  source 1..17: mol_type = other DNA
tgggtaaaccttggggc

SEQ ID NO: 15 - DNA, 58 bp, synthetic construct
  source 1..58: mol_type = other DNA
ggatccattcgttacctggctctcgccagtcgggatcctccaccaaacgtaatgcggg

SEQ ID NO: 16 - DNA, 59 bp, synthetic construct
  source 1..59: mol_type = other DNA
ttggggccgacgttgttttgatcgcgccccactgcgttctccattctggttactgccag

SEQ ID NO: 17 - DNA, 10 bp, synthetic construct
  source 1..10: mol_type = other DNA
tatcagacat

SEQ ID NO: 18 - DNA, 130 bp, Severe acute respiratory syndrome coronavirus 2
  source 1..130: mol_type = genomic DNA
  primer_bind 14..33: note = SARS-CoV-2 PCR primer 1 binding region
  misc_binding 16..37: bound_moiety = SARS-CoV-2 target promoter probe binding region
  misc_binding 38..57: bound_moiety = SARS-CoV-2 target reporter probe binding region
  primer_bind 62..85: note = SARS-CoV-2 PCR primer 2 binding region
atgtctgataatggaccccaaaatcagcgaaatgcaccccgcattacgtttggtggaccctcagattcaactggcagtaaccagaatggagaacgcagtggggcgcgatcaaaacaacgtcggccccaag

SEQ ID NO: 19 - DNA, 20 bp, synthetic construct
  source 1..20: mol_type = other DNA
gaccccaaaatcagcgaaat

SEQ ID NO: 20 - DNA, 24 bp, synthetic construct
  source 1..24: mol_type = other DNA
tctggttactgccagttgaatctg

SEQ ID NO: 21 - DNA, 86 bp, synthetic construct
  source 1..86: mol_type = other DNA
  misc_binding 1: bound_moiety = Phosphate
ttctatttcctgagcgtctgagatccctatagtgagtcgtattaatttcgcgacaacacgcgaaattaatacgactcactataggg

SEQ ID NO: 22 - DNA, 85 bp, synthetic construct
  source 1..85: mol_type = other DNA
gtatgtgggagcccacactctactcgacagatacgaatatctggacccgaccgtctcccacatacggcaggatagttcagacggt

SEQ ID NO: 23 - DNA, 86 bp, synthetic construct
  source 1..86: mol_type = other DNA
  misc_binding 1: bound_moiety = Phosphate
ctctatttcctgagcgtctgagatccctatagtgagtcgtattaatttcgcgacaacacgcgaaattaatacgactcactataggg

SEQ ID NO: 24 - DNA, 85 bp, synthetic construct; identical to SEQ ID NO: 22
  source 1..85: mol_type = other DNA

SEQ ID NO: 25 - DNA, 53 bp, synthetic construct
  source 1..53: mol_type = other DNA
ttatgtaaaggatgcgtagggatgggagggcgatgaggactaggatgatggcg

SEQ ID NO: 26 - DNA, 48 bp, synthetic construct
  source 1..48: mol_type = other DNA
ttatgtaaaggatgcgtagggatgggagggcgatgaggactaggatga

SEQ ID NO: 27 - DNA, 53 bp, synthetic construct
  source 1..53: mol_type = other DNA
gttagtattagttagttttgttgtgagtgttaggaaaagggcatacaggacta

SEQ ID NO: 28 - DNA, 150 bp, Homo sapiens
  source 1..150: mol_type = genomic DNA
tagtcctgtatgcccttttcctaacactcacaacaaaactaactaatactaacatctcagacgctcaggaaatagaaaccgtctgaactatcctgcccgccatcatcctagtcctcatcgccctcccatccctacgcatcctttacataa

SEQ ID NO: 29 - DNA, 150 bp, synthetic construct
  source 1..150: mol_type = other DNA
tagtcctgtatgcccttttcctaacactcacaacaaaactaactaatactaacatctcagacgctcaggaaatagagaccgtctgaactatcctgcccgccatcatcctagtcctcatcgccctcccatccctacgcatcctttacataa

SEQ ID NO: 30 - DNA, 83 bp, synthetic construct
  source 1..83: mol_type = other DNA
tagtcctgtatgcccttttcctaacactcacaacaaaactaactaatactaacatctcagacgctcaggaaatagaaaccgtc

SEQ ID NO: 31 - DNA, 89 bp, synthetic construct
  source 1..89: mol_type = other DNA
ttatgtaaaggatgcgtagggatgggagggcgatgaggactaggatgatggcgggcaggatagttcagacggtttctatttcctgagcg

SEQ ID NO: 32 - DNA, 88 bp, synthetic construct
  source 1..88: mol_type = other DNA
tagtcctgtatgcccttttcctaacactcacaacaaaactaactaatactaacatctcagacgctcaggaaatagagaccgtctgaac

SEQ ID NO: 33 - DNA, 87 bp, synthetic construct
  source 1..87: mol_type = other DNA
ttatgtaaaggatgcgtagggatgggagggcgatgaggactaggatgatggcgggcaggatagttcagacggtctctatttcctgag

SEQ ID NO: 34 - DNA, 26 bp, synthetic construct
  source 1..26: mol_type = other DNA
tagtcctgtatgcccttttcctaaca

SEQ ID NO: 35 - DNA, 25 bp, synthetic construct
  source 1..25: mol_type = other DNA
ttatgtaaaggatgcgtagggatgg

SEQ ID NO: 36 - DNA, 79 bp, synthetic construct
  source 1..79: mol_type = other DNA
  misc_binding 1: bound_moiety = Phosphate
atcccacaccctggaggccctatagtgagtcgtattaatttcgcgacaacacgcgaaattaatacgactcactataggg

SEQ ID NO: 37 - DNA, 89 bp, synthetic construct
  source 1..89: mol_type = other DNA
gtatgtgggagcccacactctactcgacagatacgaatatctggacccgaccgtctcccacatacgtacctaaaaggaaatctcacccc

SEQ ID NO: 38 - DNA, 79 bp, synthetic construct; identical to SEQ ID NO: 36
  source 1..79: mol_type = other DNA
  misc_binding 1: bound_moiety = Phosphate

SEQ ID NO: 39 - DNA, 89 bp, synthetic construct
  source 1..89: mol_type = other DNA
gtatgtgggagcccacactctactcgacagatacgaatatctggacccgaccgtctcccacatacgtacctaaaaggaaatctcaccct

SEQ ID NO: 40 - DNA, 58 bp, synthetic construct
  source 1..58: mol_type = other DNA
ttgtcaagtctctgctggcccagccaaaccctgtctgacaacctcttggtgaacctta

SEQ ID NO: 41 - DNA, 43 bp, synthetic construct
  source 1..43: mol_type = other DNA
ttgtcaagtctctgctggcccagccaaaccctgtctgacaacc

SEQ ID NO: 42 - DNA, 41 bp, synthetic construct
  source 1..41: mol_type = other DNA
ttgtatatgatgatctggatccaccaagacttgttttatgc

SEQ ID NO: 43 - DNA, 46 bp, synthetic construct
  source 1..46: mol_type = other DNA
atctcttgtatatgatgatctggatccaccaagacttgttttatgc

SEQ ID NO: 44 - DNA, 150 bp, Homo sapiens
  source 1..150: mol_type = genomic DNA
gcataaaacaagtcttggtggatccagatcatcatatacaagagatgaaatcctccagggtgtgggatggggtgagatttccttttaggtactaaggttcaccaagaggttgtcagacagggtttggctgggccagcagagacttgacaa

SEQ ID NO: 45 - DNA, 150 bp, synthetic construct
  source 1..150: mol_type = other DNA
gcataaaacaagtcttggtggatccagatcatcatatacaagagatgaaatcctccagggtgtgggatagggtgagatttccttttaggtactaaggttcaccaagaggttgtcagacagggtttggctgggccagcagagacttgacaa

SEQ ID NO: 46 - DNA, 81 bp, synthetic construct
  source 1..81: mol_type = other DNA
gcataaaacaagtcttggtggatccagatcatcatatacaagagatgaaatcctccagggtgtgggatggggtgagatttc

SEQ ID NO: 47 - DNA, 89 bp, synthetic construct
  source 1..89: mol_type = other DNA
ttgtcaagtctctgctggcccagccaaaccctgtctgacaacctcttggtgaaccttagtacctaaaaggaaatctcaccccatcccac

SEQ ID NO: 48 - DNA, 88 bp, synthetic construct
  source 1..88: mol_type = other DNA
gcataaaacaagtcttggtggatccagatcatcatatacaagagatgaaatcctccagggtgtgggatagggtgagatttccttttag

SEQ ID NO: 49 - DNA, 87 bp, synthetic construct
  source 1..87: mol_type = other DNA
ttgtcaagtctctgctggcccagccaaaccctgtctgacaacctcttggtgaaccttagtacctaaaaggaaatctcaccctatccc

SEQ ID NO: 50 - DNA, 24 bp, synthetic construct
  source 1..24: mol_type = other DNA
gcataaaacaagtcttggtggatc

SEQ ID NO: 51 - DNA, 20 bp, synthetic construct
  source 1..20: mol_type = other DNA
ttgtcaagtctctgctggcc

SEQ ID NO: 52 - DNA, 85 bp, synthetic construct
  source 1..85: mol_type = other DNA
  misc_binding 1: bound_moiety = Phosphate
gtcctcactgcctgtccccttccccctatagtgagtcgtattaatttcgcgacaacacgcgaaattaatacgactcactataggg

SEQ ID NO: 53 - DNA, 89 bp, synthetic construct
  source 1..89: mol_type = other DNA
gtatgtgggagcccacactctactcgacagatacgaatatctggacccgaccgtctcccacatacgtgtggggagctgtcacatccagg

SEQ ID NO: 54 - DNA, 85 bp, synthetic construct; identical to SEQ ID NO: 52
  source 1..85: mol_type = other DNA
  misc_binding 1: bound_moiety = Phosphate

SEQ ID NO: 55 - DNA, 89 bp, synthetic construct
  source 1..89: mol_type = other DNA
gtatgtgggagcccacactctactcgacagatacgaatatctggacccgaccgtctcccacatacgtgtggggagctgtcacatccagt

SEQ ID NO: 56 - DNA, 42 bp, synthetic construct
  source 1..42: mol_type = other DNA
tgtctttcctgcctgagctgacctgggcaggtcggctgtggg

SEQ ID NO: 57 - DNA, 52 bp, synthetic construct
  source 1..52: mol_type = other DNA
tgtctttcctgcctgagctgacctgggcaggtcggctgtggggtcctgtggt

SEQ ID NO: 58 - DNA, 36 bp, synthetic construct
  source 1..36: mol_type = other DNA
tatgatgatctggatccaccaagacttgttttatgc

SEQ ID NO: 59 - DNA, 150 bp, Homo sapiens
  source 1..150: mol_type = genomic DNA
cgccgatccacacggagtacttgcgctcaggaggagcaatgatctgaggagggaaggggacaggcagtgaggaccctggatgtgacagctccccacacaccacaggaccccacagccgacctgcccaggtcagctcaggcaggaaagaca

SEQ ID NO: 60 - DNA, 150 bp, synthetic construct
  source 1..150: mol_type = other DNA
cgccgatccacacggagtacttgcgctcaggaggagcaatgatctgaggagggaaggggacaggcagtgaggacactggatgtgacagctccccacacaccacaggaccccacagccgacctgcccaggtcagctcaggcaggaaagaca

SEQ ID NO: 61 - DNA, 84 bp, synthetic construct
  source 1..84: mol_type = other DNA
cgccgatccacacggagtacttgcgctcaggaggagcaatgatctgaggagggaaggggacaggcagtgaggaccctggatgtg

SEQ ID NO: 62 - DNA, 86 bp, synthetic construct
  source 1..86: mol_type = other DNA
tgtctttcctgcctgagctgacctgggcaggtcggctgtggggtcctgtggtgtgtggggagctgtcacatccagggtcctcactg

SEQ ID NO: 63 - DNA, 88 bp, synthetic construct; identical to SEQ ID NO: 48
  source 1..88: mol_type = other DNA

SEQ ID NO: 64 - DNA, 87 bp, synthetic construct; identical to SEQ ID NO: 49
  source 1..87: mol_type = other DNA

SEQ ID NO: 65 - DNA, 24 bp, synthetic construct
  source 1..24: mol_type = other DNA
gcataaaacaagtcttggtggatc

SEQ ID NO: 66 - DNA, 20 bp, synthetic construct
  source 1..20: mol_type = other DNA
ttgtcaagtctctgctggcc